European Patent Specification EP 3 594 333 B1, published November 1, 2023. Title: ENGINEERED CLEAVAGE HALF-DOMAINS. Applicant: Sangamo Therapeutics, Inc. Application EP 11740153.9. The sequence listing filed with the application follows.

SEQUENCE LISTING (56 sequences)

SEQ ID NO: 1 - protein, 7 aa, Artificial Sequence
  Synthetic peptide
RSDHLST

SEQ ID NO: 2 - protein, 7 aa, Artificial Sequence
  Synthetic peptide
TSANLSR

SEQ ID NO: 3 - protein, 7 aa, Artificial Sequence
  Synthetic peptide
RSDNLSE

SEQ ID NO: 4 - protein, 7 aa, Artificial Sequence
  Synthetic peptide
TSGSLTR

SEQ ID NO: 5 - protein, 7 aa, Artificial Sequence
  Synthetic peptide
QSGALAR

SEQ ID NO: 6 - protein, 7 aa, Artificial Sequence
  Synthetic peptide
RSDNLTR

SEQ ID NO: 7 - protein, 7 aa, Artificial Sequence
  Synthetic peptide
QSGNLAR

SEQ ID NO: 8 - protein, 7 aa, Artificial Sequence
  Synthetic peptide
QSGHLQR

SEQ ID NO: 9 - protein, 7 aa, Artificial Sequence
  Synthetic peptide
QSSDLRR

SEQ ID NO: 10 - protein, 7 aa, Artificial Sequence
  Synthetic peptide
RSDTLSE

SEQ ID NO: 11 - protein, 7 aa, Artificial Sequence
  Synthetic peptide
RSDNLSR

SEQ ID NO: 12 - protein, 7 aa, Artificial Sequence
  Synthetic peptide
QNAHRTT

SEQ ID NO: 13 - protein, 7 aa, Artificial Sequence
  Synthetic peptide
QSSNLAR

SEQ ID NO: 14 - protein, 7 aa, Artificial Sequence
  Synthetic peptide
RSDDLTR

SEQ ID NO: 15 - protein, 7 aa, Artificial Sequence
  Synthetic peptide
DRSHLSR

SEQ ID NO: 16 - protein, 7 aa, Artificial Sequence
  Synthetic peptide
DNPNLNR

SEQ ID NO: 17 - protein, 7 aa, Artificial Sequence
  Synthetic peptide
RSDDLSR

SEQ ID NO: 18 - protein, 7 aa, Artificial Sequence
  Synthetic peptide
RNAHRIN

SEQ ID NO: 19 - protein, 7 aa, Artificial Sequence
  Synthetic peptide
RSANLTR

SEQ ID NO: 20 - protein, 7 aa, Artificial Sequence
  Synthetic peptide
ASKTRKN

SEQ ID NO: 21 - protein, 7 aa, Artificial Sequence
  Synthetic peptide
DRSNLSR

SEQ ID NO: 22 - protein, 7 aa, Artificial Sequence
  Synthetic peptide
RSDHLSA

SEQ ID NO: 23 - protein, 7 aa, Artificial Sequence
  Synthetic peptide
QSGHLSR

SEQ ID NO: 24 - protein, 7 aa, Artificial Sequence
  Synthetic peptide
TSGSLSR

SEQ ID NO: 25 - protein, 7 aa, Artificial Sequence
  Synthetic peptide
RSDTLSA

SEQ ID NO: 26 - protein, 7 aa, Artificial Sequence
  Synthetic peptide
DNSNRIK

SEQ ID NO: 27 - protein, 7 aa, Artificial Sequence
  Synthetic peptide
RSAALSR

SEQ ID NO: 28 - protein, 7 aa, Artificial Sequence
  Synthetic peptide
QSGDLTR

SEQ ID NO: 29 - protein, 7 aa, Artificial Sequence
  Synthetic peptide
RSDSLSA

SEQ ID NO: 30 - protein, 7 aa, Artificial Sequence
  Synthetic peptide
DRSNLTR

SEQ ID NO: 31 - protein, 7 aa, Artificial Sequence
  Synthetic peptide
RSDNLSQ

SEQ ID NO: 32 - protein, 7 aa, Artificial Sequence
  Synthetic peptide
ASNDRKK

SEQ ID NO: 33 - protein, 7 aa, Artificial Sequence
  Synthetic peptide
DSSTRKK

SEQ ID NO: 34 - protein, 7 aa, Artificial Sequence
  Synthetic peptide
RSDNLSV

SEQ ID NO: 35 - protein, 7 aa, Artificial Sequence
  Synthetic peptide
DRSHLAR

SEQ ID NO: 36 - protein, 7 aa, Artificial Sequence
  Synthetic peptide
QRSNLVR

SEQ ID NO: 37 - protein, 7 aa, Artificial Sequence
  Synthetic peptide
QSSDLTR

SEQ ID NO: 38 - protein, 7 aa, Artificial Sequence
  Synthetic peptide
GNVDLIE

SEQ ID NO: 39 - protein, 7 aa, Artificial Sequence
  Synthetic peptide
RSSNLSR

SEQ ID NO: 40 - protein, 7 aa, Artificial Sequence
  Synthetic peptide
RSDSLSV

SEQ ID NO: 41 - protein, 7 aa, Artificial Sequence
  Synthetic peptide
TNHNRKT

SEQ ID NO: 42 - DNA, 28 bp, Artificial Sequence
  Synthetic oligonucleotide
ttgttcaggattggacacaacatcctag

SEQ ID NO: 43 - DNA, 28 bp, Artificial Sequence
  Synthetic oligonucleotide
cagctggagaagaacgaggagacggtaa

SEQ ID NO: 44 - DNA, 28 bp, Artificial Sequence
  Synthetic oligonucleotide
ctgcggatagtgaggttccggttcccat

SEQ ID NO: 45 - DNA, 28 bp, Artificial Sequence
  Synthetic oligonucleotide
tgaggaaggaggacgaaggcctctacac

SEQ ID NO: 46 - DNA, 28 bp, Artificial Sequence
  Synthetic oligonucleotide
atgatgacgcccaggagcttcaccaccc

SEQ ID NO: 47 - DNA, 28 bp, Artificial Sequence
  Synthetic oligonucleotide
gaggaagggaagtactccctggtgatgg

SEQ ID NO: 48 - DNA, 28 bp, Artificial Sequence
  Synthetic oligonucleotide
gtgcagtgaaccaggctgttctgtggct

SEQ ID NO: 49 - DNA, 28 bp, Artificial Sequence
  Synthetic oligonucleotide
gttcccagggacttgggatgggtcctgt

SEQ ID NO: 50 - DNA, 28 bp, Artificial Sequence
  Synthetic oligonucleotide
aaggaggcaaggccgaggtctgcgatct

SEQ ID NO: 51 - DNA, 28 bp, Artificial Sequence
  Synthetic oligonucleotide
aagatgtggagcaaactgaataatgaag

SEQ ID NO: 52 - DNA, 843 bp, Artificial Sequence
  Synthetic oligonucleotide
ggaagttaaagcccatgtttctaatacaatgaacattatgttatgcccaaacttaacaccatcatttcatatgatagcactttcttatagtgttaccttatgctccctgaccaaactcccagacatcaacttgtacttttctattttattctagatctttttgtattgttgttttaaatactttcctgcccattagaggacctaggagccaccctcctctcccctcttaactgatatttagcctttcatgggctttgcatataatggaaatttcaaaatccaccctgagaaatgaaaaccaagtagaggaaaaataaactcttcaaaacacacactaccttccactgctcttttgaagaaaactttacagcttccacaagttaagactccataatgacatcctgaagcttcatcagagcacaccaggcagagtttgggaggtggtcctgttgttgaggcatccagtccagacgggatccagccatactcactgctgttgaggagctggatggaggagagcttacatctggtctcatgctggggctaaagaaggggaagaacagtgttatgatttaactgtcaaaggaatatcaaaatacagttctcttagcttctcacttcatagtcagaatgctcacagtgaactctggcttcaagtgctagcaggcactaaaatatcctagctaaatatattcaaatcatgttatattcttctttaaacaaaattaagaatgaggtcatttcttttgaagtgtctccaaaatagaatggtgtggttctggttcacttcttcttctttttttttttttttttagatgcttaggatttatttttataatcacg

SEQ ID NO: 53 - DNA, 32 bp, Artificial Sequence
  Synthetic oligonucleotide
catcatcctcatcttcagccacctgtgggcgg

SEQ ID NO: 54 - DNA, 32 bp, Artificial Sequence
  Synthetic oligonucleotide
ggcaatactcatcttcactgacctgagggtgg

SEQ ID NO: 55 - DNA, 31 bp, Artificial Sequence
  Synthetic oligonucleotide
actcccctacttcaacataaactgcaaaagg

SEQ ID NO: 56 - DNA, 31 bp, Artificial Sequence
  Synthetic oligonucleotide
agacaccttcaactgcttaaactgaaaaagg